European Patent Specification EP 2 958 571 B1, published April 10, 2024. Title: DNA hypomethylating agents for cancer therapy. Applicant: MAIO, Michele CORAL, Sandra COVRE, Alessia. The sequence listing filed with the application follows.

SEQUENCE LISTING (8 sequences)

SEQ ID NO: 1 - DNA, 17 bp, Artificial Sequence
  synthetic primer
ggtgccggagctgagga

SEQ ID NO: 2 - DNA, 23 bp, Artificial Sequence
  synthetic primer
tagacaccaggaaattagggtcg

SEQ ID NO: 3 - DNA, 20 bp, Artificial Sequence
  synthetic primer
accagttcgccatggatgac

SEQ ID NO: 4 - DNA, 16 bp, Artificial Sequence
  synthetic primer
tgccggagccgttgtc

SEQ ID NO: 5 - DNA, 29 bp, Artificial Sequence
  synthetic primer
ttaagtgcgttattacgtttggtttttac

SEQ ID NO: 6 - DNA, 30 bp, Artificial Sequence
  synthetic primer
ataaccgattatttaatacaaaaatcgacg

SEQ ID NO: 7 - DNA, 31 bp, Artificial Sequence
  synthetic primer
gattaagtgtgttattatgtttggtttttat

SEQ ID NO: 8 - DNA, 32 bp, Artificial Sequence
  synthetic primer
acataaccaattatttaatacaaaaatcaaca